European Patent Specification EP 4 085 076 B1, published February 18, 2026. Title: ANTIBODIES BINDING BCMA AND USES THEREOF. Applicant: Biosion Inc. The sequence listing filed with the application follows.

SEQUENCE LISTING (25 sequences)

SEQ ID NO: 1 - protein, 5 aa, Artificial Sequence
  VH CDR1 for mouse, chimeric and humanized B1H2
NYVMH

SEQ ID NO: 2 - protein, 17 aa, Artificial Sequence
  VH CDR2 for mouse, chimeric and humanized B1H2
FIIPFNDGTKYNEHFKG

SEQ ID NO: 3 - protein, 9 aa, Artificial Sequence
  VH CDR3 for mouse, chimeric and humanized B1H2
YDFEGYFDV

SEQ ID NO: 4 - protein, 11 aa, Artificial Sequence
  VL CDR1 for mouse, chimeric and humanized B1H2
SASQDITNFLN

SEQ ID NO: 5 - protein, 7 aa, Artificial Sequence
  VL CDR2 for mouse, chimeric and humanized B1H2
STSRLHS

SEQ ID NO: 6 - protein, 9 aa, Artificial Sequence
  VL CDR3 for mouse, chimeric and humanized B1H2
QQYSNLPWT

SEQ ID NO: 7 - protein, 118 aa, Artificial Sequence
  VH for mouse and chimeric B1H2
EVQLQQSGPELVKPGASVKMSCKASGYTLTNYVMHWMKQKPGQGLEWIGFIIPFNDGTKYNEHFKGKATLTSDKSSNTAYMVLSSLTSEDSAVYYCARYDFEGYFDVWGAGTTVTVSS

SEQ ID NO: 8 - protein, 118 aa, Artificial Sequence
  VH for huB1H2-V1, huB1H2-V7, huB1H2-V13, and huB1H2-V19
EVQLVQSGAEVKKPGSSVKVSCKASGYTLTNYVMHWMRQAPGQGLEWIGFIIPFNDGTKYNEHFKGRATLTSDKSTNTAYMELSSLRSEDTAVYYCARYDFEGYFDVWGAGTLVTVSS

SEQ ID NO: 9 - protein, 118 aa, Artificial Sequence
  VH for huB1H2-V2 to huB1H2-V6, huB1H2-V8 to huB1H2-V12, huB1H2-V14 to huB1H2-V18, huB1H2-V20 to huB1H2-V24, and huB1H2-V33
  misc_feature (37)..(37): Xaa can be Val or Met
  misc_feature (72)..(72): Xaa can be Arg or Ser
  misc_feature (74)..(74): Xaa can be Thr or Lys
QVQLVQSGAEVKKPGASVKVSCKASGYTLTNYVMHWXRQAPGQGLEWIGFIIPFNDGTKYNEHFKGRVTITXDXSISTAYMQLSSLRSEDTAVYYCARYDFEGYFDVWGQGTLVTVSS

SEQ ID NO: 10 - protein, 107 aa, Artificial Sequence
  VL for mouse and chimeric B1H2
DIQMTQTTSSLSASLGDRVTISCSASQDITNFLNWYQQKPDGTVKLLIYSTSRLHSGVPSRFSGSGSGTDYSLTISNLEPEDIATYYCQQYSNLPWTFGGGTNLEIK

SEQ ID NO: 11 - protein, 107 aa, Artificial Sequence
  VL for huB1H2-V1 to huB1H2-V24 and huB1H2-V33
  misc_feature (43)..(43): Xaa can be Thr or Ala
  misc_feature (44)..(44): Xaa can be Val or Pro
  misc_feature (71)..(71): Xaa can be Tyr or Phe
  misc_feature (73)..(73): Xaa can be Phe or Leu
DIQMTQSPSSLSASVGDRVTITCSASQDITNFLNWYQQKPGKXXKLLIYSTSRLHSGVPSRFSGSGSGTDXTXTISSLQPEDIATYYCQQYSNLPWTFGQGTKVEIK

SEQ ID NO: 12 - protein, 330 aa, Artificial Sequence
  Heavy chain constant region for chimeric and humanized antibodies
ASTKGPSVFPLAPSSKSTSGGTAALGCLVKDYFPEPVTVSWNSGALTSGVHTFPAVLQSSGLYSLSSVVTVPSSSLGTQTYICNVNHKPSNTKVDKKVEPKSCDKTHTCPPCPAPELLGGPSVFLFPPKPKDTLMISRTPEVTCVVVDVSHEDPEVKFNWYVDGVEVHNAKTKPREEQYNSTYRVVSVLTVLHQDWLNGKEYKCKVSNKALPAPIEKTISKAKGQPREPQVYTLPPSREEMTKNQVSLTCLVKGFYPSDIAVEWESNGQPENNYKTTPPVLDSDGSFFLYSKLTVDKSRWQQGNVFSCSVMHEALHNHYTQKSLSLSPGK

SEQ ID NO: 13 - protein, 107 aa, Artificial Sequence [sequence omitted]

SEQ ID NO: 14 - protein, 451 aa, Artificial Sequence
  Heavy chain of BCMA BM1
QVQLVQSGAEVKKPGSSVKVSCKASGGTFSNYWMHWVRQAPGQGLEWMGATYRGHSDTYYNQKFKGRVTITADKSTSTAYMELSSLRSEDTAVYYCARGAIYDGYDVLDNWGQGTLVTVSSASTKGPSVFPLAPSSKSTSGGTAALGCLVKDYFPEPVTVSWNSGALTSGVHTFPAVLQSSGLYSLSSVVTVPSSSLGTQTYICNVNHKPSNTKVDKKVEPKSCDKTHTCPPCPAPELLGGPSVFLFPPKPKDTLMISRTPEVTCVVVDVSHEDPEVKENWYVDGVEVHNAKTKPREEQYNSTYRVVSVLTVLHQDWLNGKEYKCKVSNKALPAPIEKTISKAKGQPREPQVYTLPPSRDELTKNQVSLTCLVKGFYPSDIAVEWESNGQPENNYKTTPPVLDSDGSFFLYSKLTVDKSRWQQGNVFSCSVMHEALHNHYTQKSLSLSPGK

SEQ ID NO: 15 - protein, 214 aa, Artificial Sequence
  Light chain of BCMA BM1
DIQMTQSPSSLSASVGDRVTITCSASQDISNYLNWYQQKPGKAPKLLIYYTSNLHSGVPSRFSGSGSGTDFTLTISSLQPEDFATYYCQQYRKLPWTFGQGTKLEIKRTVAAPSVFIFPPSDEQLKSGTASVVCLLNNFYPREAKVQWKVDNALQSGNSQESVTEQDSKDSTYSLSSTLTLSKADYEKHKVYACEVTHQGLSSPVTKSFNRGEC

SEQ ID NO: 16 - protein, 184 aa, Homo sapiens
MLQMAGQCSQNEYFDSLLHACIPCQLRCSSNTPPLTCQRYCNASVTNSVKGTNAILWTCLGLSLIISLAVFVLMFLLRKINSEPLKDEFKNTGSGLLGMANIDLEKSRTGDEIILPRGLEYTVEECTCEDCIKSKPKVDSDHCFPLPAMEEGATILVTTKTNDYCKSLPAALSATEIEKSISAR

SEQ ID NO: 17 - DNA, 354 bp, Artificial Sequence
  VH for mouse B1H2
gaggtccagttgcagcagtctggacctgagctggtaaagcctggggcttcagtgaagatgtcctgcaaggcttctggatacacattaactaactatgttatgcactggatgaaacagaagcctgggcagggccttgagtggattggatttattattcctttcaatgatggtactaaatacaatgagcacttcaaaggcaaggccacactgacttcagacaaatcctccaacacagcctacatggttctcagcagcctgacctctgaggactctgcggtctattactgtgcaaggtatgatttcgagggttacttcgatgtctggggcgcagggaccacggtcaccgtctcctca

SEQ ID NO: 18 - DNA, 354 bp, Artificial Sequence
  VH for huB1H2-V4, huB1H2-V10, huB1H2-V16, huB1H2-V22, and huB1H2-V33
caggtgcagctggtgcagagcggcgccgaggtgaagaagcctggcgcctccgtgaaggtgagctgcaaggccagcggctacacactgacaaattacgtgatgcactgggtgagacaggcccctggccagggcctggagtggatcggattcatcatccccttcaacgatggcaccaagtacaatgagcacttcaagggcagagtgaccatcaccagcgatacctccatctccaccgcctacatgcagctgtccagcctgaggtccgaggataccgccgtgtactactgcgccaggtacgacttcgagggctacttcgacgtgtggggccagggcaccctggtgaccgtgtccagc

SEQ ID NO: 19 - DNA, 321 bp, Artificial Sequence
  VL for mouse B1H2
gatatccagatgacacagactacatcctccctgtctgcctctctgggagacagagtcaccatcagttgcagtgcaagtcaggacattaccaattttttaaactggtatcagcagaaaccagatggaactgttaaactcctgatctattccacatcaagattacactcaggagtcccatcaaggttcagtggcagtgggtctgggacagattattctctcaccatcagcaacctggaacctgaagatattgccacttactattgtcagcagtatagtaaccttccgtggacgttcggtggcggcaccaacctggaaatcaaa

SEQ ID NO: 20 - DNA, 321 bp, Artificial Sequence
  VL for huB1H2-V33
gacatccagatgacacagagcccctccagcctgagcgccagcgtgggagatagggtgaccatcacctgtagcgcctcccaggatatcaccaacttcctgaattggtatcaacagaagcccggcaaggcccccaagctgctgatctactccacctccagactgcacagcggcgtgccttccaggttcagcggctccggctccggcacagacttcaccttcaccatctccagcctgcagcctgaggatatcgccacctactactgccagcagtacagcaatctgccctggaccttcggccagggcaccaaggtggagatcaag

SEQ ID NO: 21 - DNA, 993 bp, Artificial Sequence
  Heavy chain constant region for chimeric and humanized antibodies
gctagcaccaagggcccatcggtcttccccctggcaccctcctccaagagcacctctgggggcacagcggccctgggctgcctggtcaaggactacttccccgaaccggtgacggtgtcgtggaactcaggcgccctgaccagcggcgtgcacaccttcccggctgtcctacagtcctcaggactctactccctcagcagcgtggtgaccgtgccctccagcagcttgggcacccagacctacatctgcaacgtgaatcacaagcccagcaacaccaaggtggacaagaaagttgagcccaaatcttgtgacaaaactcacacatgcccaccgtgcccagcacctgaactcctggggggaccgtcagtcttcctcttccccccaaaacccaaggacaccctcatgatctcccggacccctgaggtcacatgcgtggtggtggacgtgagccacgaagaccctgaggtcaagttcaactggtacgtggacggcgtggaggtgcataatgccaagacaaagccgcgggaggagcagtacaacagcacgtaccgtgtggtcagcgtcctcaccgtcctgcaccaggactggctgaatggcaaggagtacaagtgcaaggtctccaacaaagccctcccagcccccatcgagaaaaccatctccaaagccaaagggcagccccgagaaccacaggtgtacaccctgcccccatcccgggaggagatgaccaagaaccaggtcagcctgacctgcctggtcaaaggcttctatcccagcgacatcgccgtggagtgggagagcaatgggcagccggagaacaactacaagaccacgcctcccgtgctggactccgacggctccttcttcctctacagcaagctcaccgtggacaagagcaggtggcagcaggggaacgtcttctcatgctccgtgatgcatgaggctctgcacaaccactacacgcagaagagcctctccctgtctccgggtaaatga

SEQ ID NO: 22 - DNA, 324 bp, Artificial Sequence
  Light chain constant region for chimeric and humanized antibodies
cgtacggtggcggcgccatctgtcttcatcttcccgccatctgatgagcagttgaaatctggaactgcctctgttgtgtgcctgctgaataacttctatcccagagaggccaaagtacagtggaaggtggataacgccctccaatcgggtaactcccaggagagtgtcacagagcaggacagcaaggacagcacctacagcctcagcagcaccctgacgctgagcaaagcagactacgagaaacacaaagtctacgcctgcgaagtcacccatcagggcctgagctcgcccgtcacaaagagcttcaacaggggagagtgttga

SEQ ID NO: 23 - protein, 594 aa, Artificial Sequence
  Recombinant protein DT3C
MGADDVVDSSKSFVMENFSSYHGTKPGYVDSIQKGIQKPKSGTQGNYDDDWKGFYSTDNKYDAAGYSVDNENPLSGKAGGVVKVTYPGLTKVLALKVDNAETIKKELGLSLTEPLMEQVGTEEFIKRFGDGASRVVLSLPFAEGSSSVEYINNWEQAKALSVELEINFETRGKRGQDAMYEYMAQACAGNRVRRSVGSSLSCINLDWDVIRDKTKTKIESLKEHGPIKNKMSESPNKTVSEEKAKQYLEEFHQTALEHPELSELKTVTGTNPVFAGANYAAWAVNVAQVIDSETADNLEKTTAALSILPGIGSVMGIADGAVHHNTEEIVAQSIALSSLMVAQAIPLVGELVDIGFAAYNFVESIINLFQVVHNSYNRPAYSPGHKHIDEILAALPKTDTYKLILNGKTLKGETTTEAVDAATAEKVFKQYANDNGVDGEWTYDDATKTFTVTEKPEVIDASELTPAVTTYKLVINGKTLKGETTTEAVDAATAEKVFKQYANDNGVDGEWTYDDATKTFTVTEKPEVIDASELTPAVTTYKLVINGKTLKGETTTKAVDAETAEKAFKQYANDNGVDGVWTYDDATKTFTVTE

SEQ ID NO: 24 - DNA, 354 bp, Artificial Sequence
  VH for chimeric B1H2
gaggtgcagctgcagcagagcggccctgagctggtgaagcccggcgcttccgtgaagatgagctgcaaggccagcggctacacactgacaaattacgtgatgcactggatgaagcagaagcccggccagggcctggagtggatcggcttcatcatcccttttaacgacggcaccaagtacaacgagcactttaagggcaaggccacactgacatccgacaagagcagcaataccgcctacatggtgctgtccagcctgaccagcgaggactccgccgtgtactactgtgccaggtacgattttgagggctacttcgacgtgtggggcgccggcaccacagtgaccgtgagcagc

SEQ ID NO: 25 - DNA, 321 bp, Artificial Sequence
  VL for chimeric B1H2
gacatccagatgacccagacaacaagcagcctgagcgcctccctgggcgacagggtgacaatctcctgcagcgccagccaggacatcacaaacttcctgaactggtatcaacagaagcccgacggcacagtgaagctgctgatctactccacatccagactgcactccggcgtgccctccaggttctccggctccggatccggcacagattactccctgaccatcagcaacctggagcctgaggacatcgccacctactactgccagcagtacagcaatctgccttggacctttggcggcggcaccaatctggagatcaag